European Patent Application EP 4 155 385 A1, published March 29, 2023. Title: Improved Production of Glycoproteins Using Manganese. Applicant: Amgen, Inc. The sequence listing filed with the application follows.

SEQUENCE LISTING (3 sequences)

SEQ ID NO: 1 - DNA, 1725 bp, Homo sapiens
gaattccctgtggaatgtgtgtcagttagggtgtggaaagtccccaggctccccagcaggcagaagtatgcaaagcatgcatctcaattagtcagcaaccaggtgtggaaagtccccaggctccccagcaggcagaagtatgcaaagcatgcatctcaattagtcagcaaccatagtcccgcccctaactccgcccatcccgcccctaactccgcccagttccgcccattctccgccccatggctgactaattttttttatttatgcagaggccgaggccgcctcggcctctgagctattccagaagtagtgaggaggcttttttggaggcctaggcttttgcaaaaagctggtcgaggaactgaaaaaccagaaagttaactggtaagtttagtctttttgtcttttatttcaggtcccggatccggtggtggtgcaaatcaaagaactgctcctcagtggatgttgcctttacttctaggcctgtacggaagtgttacttctgctctaaaagctgctgcaacaagctggtcgagatcctaggtcacccggcgcgccccaggtcgctgagggaccccggccaggcgcggagatgggggtgcacgaatgtcctgcctggctgtggcttctcctgtccctgctgtcgctccctctgggcctcccagtcctgggcgccccaccacgcctcatctgtgacagccgagtcctggagaggtacctcttggaggccaaggaggccgagaatatcacgacgggctgtaatgaaacgtgcagcttgaatgagaatatcactgtcccagacaccaaagttaatttctatgcctggaagaggatggaggtcgggcagcaggccgtagaagtctggcagggcctggccctgctgtcggaagctgtcctgcggggccaggccctgttggtcaactcttcccaggtgaatgagaccctgcagctgcatgtggataaagccgtcagtggccttcgcagcctcaccactctgcttcgggctctgggagcccagaaggaagccatctcccctccagatgcggcctcagctgctccactccgaacaatcactgctgacactttccgcaaactcttccgagtctactccaatttcctccggggaaagctgaagctgtacacaggggaggcctgcaggacaggggacagatgaccaggtgtgtccacctgggcatatccaccacctccctcaccaacattgcttgtgccacaccctcccccgccactcctgaaccccgtcgaggggctctcagctcagcgccagcctgtcccatggacactccagtgccagcaatgacatctcaggggccagaggaactgtccagagagcaactctgagatctcgaccatgggaaatgtcagagtggagaaccacaccgagtgccactgcagcacttgttattatcacaaatcctaatagtttgcagtgggccttgctgatgatggctgacttgctcaaaaggaaaattaatttgtccagtgtctatggctttgtgagataaaaccctccttttccttgccataccatttttaacctgctttgagaatatactgcagctttattgcttttctccttatcctacaatataatcagtagtcttgatcttttcatttggaatgaaatatggcatttagcatgaccataaaaagctgattccactggaaataaagtcttttaaatcatcactctatcactgaattcta

SEQ ID NO: 2 - protein, 193 aa, Homo sapiens
  mat_peptide (28)..(192)
MGVHECPAWLWLLLSLLSLPLGLPVLGAPPRLICDSRVLERYLLEAKEAENITTGCNETCSLNENITVPDTKVNFYAWKRMEVGQQAVEVWQGLALLSEAVLRGQALLVNSSQVNETLQLHVDKAVSGLRSLTTLLRALGAQKEAISPPDAASAAPLRTITADTFRKLFRVYSNFLRGKLKLYTGEACRTGDR

SEQ ID NO: 3 - protein, 193 aa, Homo sapiens
  mat_peptide (28)..(192)
MGVHECPAWLWLLLSLLSLPLGLPVLGAPPRLICDSRVLERYLLEAKEAENITTGCAEHCSLNENITVPDTKVNFYAWKRMEVGQQAVEVWQGLALLSEAVLRGQALLVNSSQPWEPLQLHVDKAVSGLRSLTTLLRALGAQKEAISPPDAASAAPLRTITADTFRKLFRVYSNFLRGKLKLYTGEACRTGDR